European Patent Application EP 4 635 979 A1, published October 22, 2025. Title: Low-Molecular-Weight Collagen Having 164.88° Triple-Helix Structure. Applicant: Shanxi Jinbo Bio-Pharmaceutical Co., Ltd. Application CN. The sequence listing filed with the application follows.

SEQUENCE LISTING (2 sequences)

SEQ ID NO: 1 - protein, 30 aa, Homo sapiens
GERGAPGFRGPAGPNGIPGEKGPAGERGAP

SEQ ID NO: 2 - DNA, 90 bp, synthetic construct
  source 1..90: mol_type = other DNA
ggagaaaggggggcgccaggcttccgcggtccggcgggtccgaacggcatcccgggtgagaagggtccggctggcgaacgtggcgcaccg